European Patent Specification EP 3 689 879 B1, published February 12, 2025. Title: HETEROCYCLIC COMPOUND. Applicant: TAKEDA PHARMACEUTICAL COMPANY LIMITED. The sequence listing filed with the application follows.

SEQUENCE LISTING (2 sequences)

SEQ ID NO: 1 - DNA, 41 bp, Artificial Sequence
  primer
ccaccatcatcacggatccatgccagaggaaagttccccca

SEQ ID NO: 2 - DNA, 40 bp, Artificial Sequence
  primer
tggtgctcgagtgcggccgctcagggtggggacgcagttc